European Patent Application EP 4 177 270 A1, published May 10, 2023. Title: Anti-cd47 agent-based ovarian cancer therapy. Applicant: FORTY SEVEN, INC. The sequence listing filed with the application follows.

SEQUENCE LISTING (2 sequences)

SEQ ID NO: 1 - protein, 444 aa, synthetic construct
  REGION 1..444: note = source = /note="Description of Artificial Sequence: Syntheticpolypeptide"
QVQLVQSGAEVKKPGASVKVSCKASGYTFTNYNMHWVRQAPGQRLEWMGTIYPGNDDTSYNQKFKDRVTITADTSASTAYMELSSLRSEDTAVYYCARGGYRAMDYWGQGTLVTVSSASTKGPSVFPLAPCSRSTSESTAALGCLVKDYFPEPVTVSWNSGALTSGVHTFPAVLQSSGLYSLSSVVTVPSSSLGTKTYTCNVDHKPSNTKVDKRVESKYGPPCPPCPAPEFLGGPSVFLFPPKPKDTLMISRTPEVTCVVVDVSQEDPEVQFNWYVDGVEVHNAKTKPREEQFNSTYRVVSVLTVLHQDWLNGKEYKCKVSNKGLPSSIEKTISKAKGQPREPQVYTLPPSQEEMTKNQVSLTCLVKGFYPSDIAVEWESNGQPENNYKTTPPVLDSDGSFFLYSRLTVDKSRWQEGNVFSCSVMHEALHNHYTQKSLSLSLGK

SEQ ID NO: 2 - protein, 219 aa, synthetic construct
  REGION 1..219: note = source = /note="Description of Artificial Sequence: Syntheticpolypeptide"
DIVMTQSPLSLPVTPGEPASISCRSSQSIVYSNGNTYLGWYLQKPGQSPQLLIYKVSNRFSGVPDRFSGSGSGTDFTLKISRVEAEDVGVYYCFQGSHVPYTFGQGTKLEIKRTVAAPSVFIFPPSDEQLKSGTASVVCLLNNFYPREAKVQWKVDNALQSGNSQESVTEQDSKDSTYSLSSTLTLSKADYEKHKVYACEVTHQGLSSPVTKSFNRGEC